European Patent Specification EP 3 997 240 B1, published July 12, 2023. Title: METHODS FOR DETERMINING THE CONCENTRATION OF A CARBAPENEM ANTIBIOTIC IN A BIOLOGICAL SAMPLE. Applicant: Université de Liège. The sequence listing filed with the application follows.

SEQUENCE LISTING (56 sequences)

SEQ ID NO: 1 - protein, 265 aa, Klebsiella pneumoniae
  PEPTIDE (1)..(22): SIGNAL PEPTIDE
MRVLALSAVFLVASIIGMPAVAKEWQENKSWNAHFTEHKSQGVVVLWNENKQQGFTNNLKRANQAFLPASTFKIPNSLIALDLGVVKDEHQVFKWDGQTRDIATWNRDHNLITAMKYSVVPVYQEFARQIGEARMSKMLHAFDYGNEDISGNVDSFWLDGGIRISATEQISFLRKLYHNKLHVSERSQRIVKQAMLTEANGDYIIRAKTGYSTRIEPKIGWWVGWVELDDNVWFFAMNMDMPTSDGLGLRQAITKEVLKQEKIIP

SEQ ID NO: 2 - protein, 265 aa, Shewanella oneidensis
  PEPTIDE (1)..(22): SIGNAL PEPTIDE
MRVLALSAVLVVASIVGMPAMANEWQEKPSWNTHFSEHKAQGVIVLWNENKQQGFTNNLKRANQAFLPASTFKIPNSLIALDLGVVKDEHQVFKWDGQTRDIAAWNRDHDLITAMKYSVVPVYQEFARQIGQARMSKMLHAFDYGNEDISGNLDSFWLDGGIRISATEQVAFLRKLYHNKLHVSERSQRIVKQAMLTEANSDYIIRAKTGYSTRIEPQIGWWVGWVELDDNVWFFAMNMDMPTADGLGLRQAITKEVLKQEKIIP

SEQ ID NO: 3 - protein, 265 aa, Klebsiella pneumoniae
  PEPTIDE (1)..(22): SIGNAL PEPTIDE
MRVLALSAVFLVASIIGMPAVAKEWQENKSWNAHFTEHKSQGVVVLWNENKQQGFTNNLKRANQAFLPASTFKIPNSLIALDLGVVKDEHQVFKWDGQTRDIATWNRDHNLITAMKYSVVPVYQEFARQIGEARMSKMLHAFDYGNEDISGNVDSFWLDGGIRISATEQISFLRKLYHNKLHVSERSQRIVKQAMLTEANGDYIIRAKTGYSARIEPKIGWWVGWVELDDNVWFFAMNMDMPTSDGLGLRQAITKEVLKQEKIIP

SEQ ID NO: 4 - protein, 261 aa, Enterobacter cloacae
  PEPTIDE (1)..(22): SIGNAL PEPTIDE
MRVLALSAVFLVASIIGMPAVAKEWQENKSWNAHFTEHKSQGVVVLWNENKQQGFTNNLKRANQAFLPASTFKIPNSLIALDLGVVKDEHQVFKWDGQTRDIATWNRDHNLITAMKYSVVPVYQEFARQIGEARMSKMLHAFDYGNEDISGNVDSFWLDGGIRISATEQISFLRKLYHNKLHVSERSQRIVKQAMLTEANGDYIIRAKTGYDTKIGWWVGWVELDDNVWFFAMNMDMPTSDGLGLRQAITKEVLKQEKIIP

SEQ ID NO: 5 - protein, 265 aa, Klebsiella pneumoniae
  PEPTIDE (1)..(22): SIGNAL PEPTIDE
MRVLALSAVFLVASIIGMPAVAKEWQENKSWNAHFTEHKSQGVVVLWNENKQQGFTNNLKRANQAFLPASTFKIPNSLIALDLGVVKDEHQVFKWDGQTRDIAAWNRDHDLITAMKYSVVPVYQEFARQIGEARMSKMLHAFDYGNEDISGNVDSFWLDGGIRISATQQIAFLRKLYHNKLHVSERSQRIVKQAMLTEANGDYIIRAKTGYSTRIEPKIGWWVGWVELDDNVWFFAMNMDMPTSDGLGLRQAITKEVLKQEKIIP

SEQ ID NO: 6 - protein, 265 aa, Shewanella xiamenensis
  PEPTIDE (1)..(22): SIGNAL PEPTIDE
MRVLALSAVFLVASIIGMPAVAKEWQENKSWNAHFTEYKSQGVVALWNENKQQGFTNNLKRANQAFLPASTFKIPNSLIALDLGVVKDEHQVFKWDGQTRDIATWNRDHNLITAMKYSVVPVYQEFARQIGEARMSKMLHAFDYGNEDISGNVGSFWLDGGIRISATEQISFLRKLYHNKLHVSERSQRIVKQAMLTEANGDYIIRAKTGYSTRIEPKIGWWVGWVELDDNVWFFAMNMDMPTSDGLGLRQAITKEVLKQEKIIP

SEQ ID NO: 7 - protein, 265 aa, Klebsiella pneumoniae
  PEPTIDE (1)..(22): SIGNAL PEPTIDE
MRVLALSAVFLVASIIGMPAVAKEWQENKSWNAHFTEHKSQGVVVLWNENKQQGFTNNLKRANQAFLPASTFKIPNSLIALDLGVVKDEHQVFKWDGHRRDIATWNRDHNLITAMKYSVVPVYQEFARQIGEARMSKMLHAFDYGNEDISGNVDSFWLDGGIRISATEQISFLRKLYHNKLHVSERSQRIVKQAMLTEANGDYIIRAKTGYSTRIEPKIGWWVGWVELDDNVWFFAMNMDMPTSDGLGLRQAITKEVLKQEKIIP

SEQ ID NO: 8 - protein, 265 aa, Klebsiella pneumoniae
  PEPTIDE (1)..(22): SIGNAL PEPTIDE
MRVLALSAVFLVASIIGMPAVAKEWQENKSWNAHFTEHKSQGVVVLWNENKQQGFTNNLKRANQAFLPASTFKIPNSLIALDLGVVKDEHQVFKWDGQTRDIATWNRDHNLITAMKYSVVPVYQEFARQIGEARMSKMLHAFDYGNEDISGNVDSFWLDGGIRISATEQISFLRKLYHNKLHVSERSQRIVKQAMLTEANGDYIIRAKTGYSTGIEPKIGWWVGWVELDDNVWFFAMNMDMPTSDGLGLRQAITKEVLKQEKIIP

SEQ ID NO: 9 - protein, 265 aa, Klebsiella pneumoniae
  PEPTIDE (1)..(22): SIGNAL PEPTIDE
MRVLALSAVFLVASIIGMPAVAKEWQENKSWNAHFTEHKSQGVVVLWNENKQQGFTNNLKRANQAFLPASTFKIPNSLIALDLGVVKDEHQVFKWDGQTRDIATWNRDHNLITAMKYSVVPVYQYFARQIGEARMSKMLHAFDYGNEDISGNVDSFWLDGGIRISATEQISFLRKLYHNKLHVSERSQRIVKQAMLTEANGDYIIRAKTGYSTRIEPKIGWWVGWVELDDNVWFFAMNMDMPTSDGLGLRQAITKEVLKQEKIIP

SEQ ID NO: 10 - protein, 261 aa, Klebsiella pneumoniae
  PEPTIDE (1)..(22): SIGNAL PEPTIDE
MRVLALSAVFLVASIIGMPAVAKEWQENKSWNAHFTEHKSQGVVVLWNENKQQGFTNNLKRANQAFLPASTFKIPNSLIALDLGVVKDEHQVFKWDGQTRDIATWNRDHNLITAMKYSVVPVYQEFARQIGEARMSKMLHAFDYGNEDISGNVDSFWLDGGIRISATEQISFLRKLYHNKLHVSERSQRIVKQAMLTEANGDYIIRAKTGSNTKIGWWVGWVELDDNVWFFAMNMDMPTSDGLGLRQAITKEVLKQEKIIP

SEQ ID NO: 11 - protein, 265 aa, Escherichia coli
  PEPTIDE (1)..(22): SIGNAL PEPTIDE
MRVLALSAVFLVASIIGMPAVAKEWQENKSWNAHFTEHKSQGVVVLWNENKQQGFTNNLKRANQAFLPASTFKIPNSLIALDLGVVKDEHQVFKWDGQTRDIAAWNRDHDLITAMKYSVVPVYQEFARQIGEARMSKMLHAFDYGNEDISGNVDSFWLDGGIRISATQQIAFLRKLYHNKLHVSERSQRIVKQAMLTEANGDYIIRAKTGYSTSIEPKIGWWVGWVELDDNVWFFAMNMDMPTSDGLGLRQAITKEVLKQEKIIP

SEQ ID NO: 12 - protein, 265 aa, Enterobacter sp. 87F-2
  PEPTIDE (1)..(22): SIGNAL PEPTIDE
MRVLALSAVFLVASIIGMPAVAKEWQENKSWNAHFTEHKSQGVVVLWNENKQQGFTNNLKRANQAFLPASTFKIPNSLIALDLGVVKDEHQVFKWDGQTRDIATWNRDHNLITAMKYSVVPVYQEFARQIGEARMSKMLHAFDYGNEDISGNVDSFWLDGGIRISATEQISFLRKLYHNKLHVSERSQRIVKQAMLTEANGDYIIRAKTGYETRIEPKIGWWVGWVELDDNVWFFAMNMDMPTSDGLGLRQAITKEVLKQEKIIP

SEQ ID NO: 13 - protein, 261 aa, Serratia marcescens
  PEPTIDE (1)..(22): SIGNAL PEPTIDE
MRVLALSAVFLVASIIGMPAVAKEWQENKSWNAHFTEHKSQGVVVLWNENKQQGFTNNLKRANQAFLPASTFKIPNSLIALDLGVVKDEHQVFKWDGQTRDIATWNRDHNLITAMKYSVVPVYQEFARQIGEARMSKMLHAFDYGNEDISGNVDSFWLDGGIRISATEQISFLRKLYHNKLHVSERSQRIVKQAMLTEANGDYIIRAKTGYSPKIGWWVGWVELDDNVWFFAMNMDMPTSDGLGLRQAITKEVLKQEKIIP

SEQ ID NO: 14 - protein, 265 aa, Shewanella xiamenensis
  PEPTIDE (1)..(22): SIGNAL PEPTIDE
MRVLALSAVFLVASIIGMPAVAKEWQENKSWNAHFTEHKSQGVVVLWNENKQQGFTNNLKRANQAFLPASTFKIPNSLIALDLGVVKDEHQVFKWDGQTRDIATWNRDHNLITAMKYSVVPVYQEFARQIGEARMSKMLHAFDYGNEDISGNLDTFWLDGGIRISATEQISFLRKLYHNKLHVSERSQRIVKQAMLTEANADYIIRAKTGYSTRIEPKIGWWVGWVELDDNVWFFAMNMDMPTSDGLGLRQAITKEVLKQEKIIP

SEQ ID NO: 15 - protein, 263 aa, Escherichia coli
  PEPTIDE (1)..(22): SIGNAL PEPTIDE
MRVLALSAVFLVASIIGMPAVAKEWQENKSWNAHFTEHKSQGVVVLWNENKQQGFTNNLKRANQAFLPASTFKIPNSLIALDLGVVKDEHQVFKWDGQTRDIATWNRDHNLITAMKYSVVPVYQEFARQIGEARMSKMLHAFDYGNEDISGNVDSFWLDGGIRISATEQISFLRKLYHNKLHVSERSQRIVKQAMLTEANGDYIIRAKTGYGYDTKIGWWVGWVELDDNVWFFAMNMDMPTSDGLGLRQAITKEVLKQEKIIP

SEQ ID NO: 16 - protein, 261 aa, Escherichia coli
  PEPTIDE (1)..(22): SIGNAL PEPTIDE
MRVLALSAVFLVASIIGMPAVAKEWQENKSWNAHFTEHKSQGVVVLWNENKQQGFTNNLKRANQAFLPASTFKIPNSLIALDLGVVKDEHQVFKWDGQTRDIATWNRDHNLITAMKYSVVPVHQEFARQIGEARMSKMLHAFDYGNEDISGNVDSFWLDGGIRISATEQISFLRKLYHNKLHVSERSQRIVKQAMLTEANGDYIIRAKTGYDTKIGWWVGWVELDDNVWFFAMNMDMPTSDGLGLRQAITKEVLKQEKIIP

SEQ ID NO: 17 - protein, 265 aa, Klebsiella pneumoniae
  PEPTIDE (1)..(22): SIGNAL PEPTIDE
MRVLALSAVFLVASIIGMPAVAKEWQENKSWNAHFTEHKSQGVVVLWNENKQQGFTNNLKRANQAFLPASTFKIPNSLIALDLGVVKDEHQVFKWDGQTRDIAAWNRDHDLITAMKYSVVPVYQEFARQIGEARMSKMLHAFDYGNEDISGNVDSFWLDGGIRISATQQIAFLRKLYHNKLHVSERSQRIVKQAMLTEANGDYIIRAKTGYSTGIEPKIGWWVGWVELDDNVWFFAMNMDMPTSDGLGLRQAITKEVLKQEKIIP

SEQ ID NO: 18 - protein, 265 aa, Enterobacter asburiae
  PEPTIDE (1)..(22): SIGNAL PEPTIDE
MRALALSAVLMVTTMIGMPAVAKEWQENKSWNAHFSEHKTQGVVVLWNENTQQGFTNDLKRANQAFLPASTFKIPNSLIALDLGVVKDEHQVFKWDGQTRDIAAWNRDHDLITAMKYSVVPVYQEFARQIGEARMSKMLHAFDYGNEDISGNLDSFWLDGGIRISATQQIAFLRKLYHNKLHVSERSQRIVKQAMLTEANADYIIRAKTGYSVRIEPKIGWWVGWIELDDNVWFFATNMDMPTAEGLGLRQTITKAVLKQEKIIP

SEQ ID NO: 19 - protein, 265 aa, Klebsiella pneumoniae
  PEPTIDE (1)..(22): SIGNAL PEPTIDE
MRVLALSTVFLVASIIGMPAVAKEWQENKSWNAHFTEHKSQGVVVLWNENKQQGFTNNLKRANQAFLPASTFKIPNSLIALDLGVVKDEHQVFKWDGQTRDIATWNRDHNLITAMKYSVVPVYQEFARQIGEARMSKMLHAFDYGNEDISGNVDSFWLDGGIRISATEQISFLRKLYHNKLHVSERSQRIVKQAMLTEANGDYIIRAKTGYSTRIEPKIGWWVGWVELDDNVWFFAMNMDMPTSDGLGLRQAITKEVLKQEKIIP

SEQ ID NO: 20 - protein, 265 aa, Shewanella sp. 10A
  PEPTIDE (1)..(22): SIGNAL PEPTIDE
MRVLALSAVFLVASIIGMPAVAKEWQENKSWNAHFTEHKSQGVVVLWNENKQQGFTNNLKRANQAFLPASTFKIPNSLIALDLGVVKDEHQVFKWDGQTRDIATWNRDHNLITAMKYSVVPVYQEFARQIGEARMSKMLHAFDYGNEDISGNLDTFWLDGGIRISATEQISFLRKLYHNKLHVSERSQRIVKQAMLTEANGDYIIRAKTGYSTRIEPKIGWWVGWVELDDNVWFFAMNMDMPTSDGLGLRQAITKEVLKQEKIIP

SEQ ID NO: 21 - protein, 265 aa, Shewanella sp. W17
  PEPTIDE (1)..(22): SIGNAL PEPTIDE
MRVLALSAVFLVASIIGMPAVAKEWQENKSWNAHFTEHKSQGVVALWNENKQQGFTNNLKRANQAFLPASTFKIPNSLIALDLGVVKDEHQVFKWDGQTRDIATWNRDHNLITAMKYSVVPVYQEFARQIGEARMSKMLHAFDYGNEDISGNVDSFWLDGGIRISATEQISFLRKLYHNKLHVSERSQRIVKQAMLTEANSDYIIRAKTGYSTRIEPKIGWWVGWVELDDNVWFFAMNMDMPTSDGLGLRQAITKEVLKQEKIIP

SEQ ID NO: 22 - protein, 263 aa, Klebsiella pneumoniae
  PEPTIDE (1)..(22): SIGNAL PEPTIDE
MRVLALSAVFLVASIIGMPAVAKEWQENKSWNAHFTEHKSQGVVVLWNENKQQGFTNNLKRANQAFLPASTFKIPNSLIALDLGVVKDEHQVFKWDGQTRDIATWNRDHNLITAMKYSVVPVYQEFARQIGEARMSKMLHAFDYGNEDISGNVDSFWLDGGIRISATEQISFLRKLYHNKLHVSERSQRIVKQAMLTEANGDYIIRAKTGYSTKPKIGWWVGWVELDDNVWFFAMNMDMPTSDGLGLRQAITKEVLKQEKIIP

SEQ ID NO: 23 - protein, 265 aa, Klebsiella pneumoniae
  PEPTIDE (1)..(22): SIGNAL PEPTIDE
MRVLALSAVFLVASIIGMPAVAKEWQENKSWNAHFTEHKSQGVVVLWNENKQQGFTNNLKRANQAFLPASTFKIPNSLIALDLGVVKDEHQVFKWDGQTRDIATWNRDHNLITAMKYSVLPVYQEFARQIGEARMSKMLHAFDYGNEDISGNVDSFWLDGGIRISATEQISFLRKLYHNKLHVSERSQRIVKQAMLTEANGDYIIRAKTGYSTRIEPKIGWWVGWVELDDNVWFFAMNMDMPTSDGLGLRQAITKEVLKQEKIIP

SEQ ID NO: 24 - protein, 265 aa, Shewanella xiamenensis
  PEPTIDE (1)..(22): SIGNAL PEPTIDE
MRVLALSAVFLVASIIGMPAVAKEWQENKSWNAHFTEHKSQGVVVLWNENKQQGFTNNLKRANQAFLPASTFKIPNSLIALDLGVVKDEHQVFKWDGQTRDIATWNRDHNLITAMKYSVVPVYQEFARQIGEARMSKMLHAFDYGNEDISGNVDSFWLDGGIRISATEQISFLRKLYHNKLHVSERSQRIVKQAMLTEANADYIIRAKTGYSGRIEPKFGWWVGWVELDDNVWFFAMNMDMPTSDGLGLRQAITKEVLKQEKIIP

SEQ ID NO: 25 - protein, 265 aa, Shewanella xiamenensis
  PEPTIDE (1)..(22): SIGNAL PEPTIDE
MRVLALSAVFLVASIIGMPAVAREWQENKSWNVHFTEHKSQGVVVLWNENKQQGFTNNLKRANQAFLPASTFKIPNSLIALDLGVVKDEHQVFKWDGQTRDIATWNRDHNLITAMKYSVVPVYQEFARQIGEARMSKMLHAFDYGNEDISGNVDSFWLDGGIRISAIEQISFLRKLYHNKLHVSERSQRIVKQAMLTEANGDYIIRAKTGYSTRIEPKIGWWVGWVELDDNVWFFAMNMDMPTSDGLGLRQAITKEVLKQEKIIP

SEQ ID NO: 26 - protein, 265 aa, Shewanella xiamenensis
  PEPTIDE (1)..(22): SIGNAL PEPTIDE
MRVLALSAVFLVASIIGMPAVAKEWQENKSWNAHFTEHKSQGVVALWNENKQQGFTNNLKRANQAFLPASTFKIPNSLIALDLGVVKDEHQVFKWDGQTRDIATWNRDHNLITAMKYSVVPVYQEFARQIGEARMSKMLHAFDYGNEDISGNVDSFWLDGGIRISAIEQISFLRKLYHNKLHVSERSQRIVKQAMLTEANGDYIIRAKTGYSTRIEPKIGWWVGWVELDDNVWFFAMNMDMPTSDGLGLRQAITKEVLKQEKIIP

SEQ ID NO: 27 - protein, 265 aa, Escherichia coli
  PEPTIDE (1)..(22): SIGNAL PEPTIDE
MRVLALSAVFLVASIIGMPAVAKEWQENKSWNAHFTEHKSQGVVVLWNENKQQGFTNNLKRANQAFLPASTFKIPNSLIALDLGVVKDEHQVFKWDGQTRDIATWNRDHNLITAMKYSVVPVYQEFARQIGEARMSKMLHDFDYGNEDISGNVDSFWLDGGIRISATEQISFLRKLYHNKLHVSERSQRIVKQAMLTEANGDYIIRAKTGYSTRIEPKIGWWVGWVELDDNVWFFAMNMDMPTSDGLGLRQAITKEVLKQEKIIP

SEQ ID NO: 28 - protein, 265 aa, Shewanella sp. FDAARGOS_354
  PEPTIDE (1)..(22): SIGNAL PEPTIDE
MRVLALSAVFLVASIIGMPAVAKEWQENKSWNAHFTEHKSQGVVALWNENKQQGFTNNLKRANQAFLPASTFKIPNSLIALDLGVVKDEHQVFKWDGQTRDIATWNRDHNLITAMKYSVVPVYQEFARQIGEARMSKMLHAFDYGNEDISGNVDSFWLDGGIRISATEQISFLRKLYHNKLHVSERSQRIVKQAMLTEANGDYIIRAKTGYSTRIEPKIGWWVGWVELDDNVWFFAMNMDMPTSDGLGLRQAITKEVLKQEKIIP

SEQ ID NO: 29 - protein, 243 aa, Klebsiella pneumoniae
KEWQENKSWNAHFTEHKSQGVVVLWNENKQQGFTNNLKRANQAFLPASTFKIPNSLIALDLGVVKDEHQVFKWDGQTRDIATWNRDHNLITAMKYSVVPVYQEFARQIGEARMSKMLHAFDYGNEDISGNVDSFWLDGGIRISATEQISFLRKLYHNKLHVSERSQRIVKQAMLTEANGDYIIRAKTGYSTRIEPKIGWWVGWVELDDNVWFFAMNMDMPTSDGLGLRQAITKEVLKQEKIIP

SEQ ID NO: 30 - protein, 243 aa, Shewanella oneidensis
NEWQEKPSWNTHFSEHKAQGVIVLWNENKQQGFTNNLKRANQAFLPASTFKIPNSLIALDLGVVKDEHQVFKWDGQTRDIAAWNRDHDLITAMKYSVVPVYQEFARQIGQARMSKMLHAFDYGNEDISGNLDSFWLDGGIRISATEQVAFLRKLYHNKLHVSERSQRIVKQAMLTEANSDYIIRAKTGYSTRIEPQIGWWVGWVELDDNVWFFAMNMDMPTADGLGLRQAITKEVLKQEKIIP

SEQ ID NO: 31 - protein, 243 aa, Klebsiella pneumoniae
KEWQENKSWNAHFTEHKSQGVVVLWNENKQQGFTNNLKRANQAFLPASTFKIPNSLIALDLGVVKDEHQVFKWDGQTRDIATWNRDHNLITAMKYSVVPVYQEFARQIGEARMSKMLHAFDYGNEDISGNVDSFWLDGGIRISATEQISFLRKLYHNKLHVSERSQRIVKQAMLTEANGDYIIRAKTGYSARIEPKIGWWVGWVELDDNVWFFAMNMDMPTSDGLGLRQAITKEVLKQEKIIP

SEQ ID NO: 32 - protein, 239 aa, Enterobacter cloacae
KEWQENKSWNAHFTEHKSQGVVVLWNENKQQGFTNNLKRANQAFLPASTFKIPNSLIALDLGVVKDEHQVFKWDGQTRDIATWNRDHNLITAMKYSVVPVYQEFARQIGEARMSKMLHAFDYGNEDISGNVDSFWLDGGIRISATEQISFLRKLYHNKLHVSERSQRIVKQAMLTEANGDYIIRAKTGYDTKIGWWVGWVELDDNVWFFAMNMDMPTSDGLGLRQAITKEVLKQEKIIP

SEQ ID NO: 33 - protein, 243 aa, Klebsiella pneumoniae
KEWQENKSWNAHFTEHKSQGVVVLWNENKQQGFTNNLKRANQAFLPASTFKIPNSLIALDLGVVKDEHQVFKWDGQTRDIAAWNRDHDLITAMKYSVVPVYQEFARQIGEARMSKMLHAFDYGNEDISGNVDSFWLDGGIRISATQQIAFLRKLYHNKLHVSERSQRIVKQAMLTEANGDYIIRAKTGYSTRIEPKIGWWVGWVELDDNVWFFAMNMDMPTSDGLGLRQAITKEVLKQEKIIP

SEQ ID NO: 34 - protein, 243 aa, Shewanella xiamenensis
KEWQENKSWNAHFTEYKSQGVVALWNENKQQGFTNNLKRANQAFLPASTFKIPNSLIALDLGVVKDEHQVFKWDGQTRDIATWNRDHNLITAMKYSVVPVYQEFARQIGEARMSKMLHAFDYGNEDISGNVGSFWLDGGIRISATEQISFLRKLYHNKLHVSERSQRIVKQAMLTEANGDYIIRAKTGYSTRIEPKIGWWVGWVELDDNVWFFAMNMDMPTSDGLGLRQAITKEVLKQEKIIP

SEQ ID NO: 35 - protein, 243 aa, Klebsiella pneumoniae
KEWQENKSWNAHFTEHKSQGVVVLWNENKQQGFTNNLKRANQAFLPASTFKIPNSLIALDLGVVKDEHQVFKWDGHRRDIATWNRDHNLITAMKYSVVPVYQEFARQIGEARMSKMLHAFDYGNEDISGNVDSFWLDGGIRISATEQISFLRKLYHNKLHVSERSQRIVKQAMLTEANGDYIIRAKTGYSTRIEPKIGWWVGWVELDDNVWFFAMNMDMPTSDGLGLRQAITKEVLKQEKIIP

SEQ ID NO: 36 - protein, 243 aa, Klebsiella pneumoniae
KEWQENKSWNAHFTEHKSQGVVVLWNENKQQGFTNNLKRANQAFLPASTFKIPNSLIALDLGVVKDEHQVFKWDGQTRDIATWNRDHNLITAMKYSVVPVYQEFARQIGEARMSKMLHAFDYGNEDISGNVDSFWLDGGIRISATEQISFLRKLYHNKLHVSERSQRIVKQAMLTEANGDYIIRAKTGYSTGIEPKIGWWVGWVELDDNVWFFAMNMDMPTSDGLGLRQAITKEVLKQEKIIP

SEQ ID NO: 37 - protein, 243 aa, Klebsiella pneumoniae
KEWQENKSWNAHFTEHKSQGVVVLWNENKQQGFTNNLKRANQAFLPASTFKIPNSLIALDLGVVKDEHQVFKWDGQTRDIATWNRDHNLITAMKYSVVPVYQYFARQIGEARMSKMLHAFDYGNEDISGNVDSFWLDGGIRISATEQISFLRKLYHNKLHVSERSQRIVKQAMLTEANGDYIIRAKTGYSTRIEPKIGWWVGWVELDDNVWFFAMNMDMPTSDGLGLRQAITKEVLKQEKIIP

SEQ ID NO: 38 - protein, 239 aa, Klebsiella pneumoniae
KEWQENKSWNAHFTEHKSQGVVVLWNENKQQGFTNNLKRANQAFLPASTFKIPNSLIALDLGVVKDEHQVFKWDGQTRDIATWNRDHNLITAMKYSVVPVYQEFARQIGEARMSKMLHAFDYGNEDISGNVDSFWLDGGIRISATEQISFLRKLYHNKLHVSERSQRIVKQAMLTEANGDYIIRAKTGSNTKIGWWVGWVELDDNVWFFAMNMDMPTSDGLGLRQAITKEVLKQEKIIP

SEQ ID NO: 39 - protein, 243 aa, Escherichia coli
KEWQENKSWNAHFTEHKSQGVVVLWNENKQQGFTNNLKRANQAFLPASTFKIPNSLIALDLGVVKDEHQVFKWDGQTRDIAAWNRDHDLITAMKYSVVPVYQEFARQIGEARMSKMLHAFDYGNEDISGNVDSFWLDGGIRISATQQIAFLRKLYHNKLHVSERSQRIVKQAMLTEANGDYIIRAKTGYSTSIEPKIGWWVGWVELDDNVWFFAMNMDMPTSDGLGLRQAITKEVLKQEKIIP

SEQ ID NO: 40 - protein, 243 aa, Enterobacter sp. 87F-2
KEWQENKSWNAHFTEHKSQGVVVLWNENKQQGFTNNLKRANQAFLPASTFKIPNSLIALDLGVVKDEHQVFKWDGQTRDIATWNRDHNLITAMKYSVVPVYQEFARQIGEARMSKMLHAFDYGNEDISGNVDSFWLDGGIRISATEQISFLRKLYHNKLHVSERSQRIVKQAMLTEANGDYIIRAKTGYETRIEPKIGWWVGWVELDDNVWFFAMNMDMPTSDGLGLRQAITKEVLKQEKIIP

SEQ ID NO: 41 - protein, 239 aa, Serratia marcescens
KEWQENKSWNAHFTEHKSQGVVVLWNENKQQGFTNNLKRANQAFLPASTFKIPNSLIALDLGVVKDEHQVFKWDGQTRDIATWNRDHNLITAMKYSVVPVYQEFARQIGEARMSKMLHAFDYGNEDISGNVDSFWLDGGIRISATEQISFLRKLYHNKLHVSERSQRIVKQAMLTEANGDYIIRAKTGYSPKIGWWVGWVELDDNVWFFAMNMDMPTSDGLGLRQAITKEVLKQEKIIP

SEQ ID NO: 42 - protein, 243 aa, Shewanella xiamenensis
KEWQENKSWNAHFTEHKSQGVVVLWNENKQQGFTNNLKRANQAFLPASTFKIPNSLIALDLGVVKDEHQVFKWDGQTRDIATWNRDHNLITAMKYSVVPVYQEFARQIGEARMSKMLHAFDYGNEDISGNLDTFWLDGGIRISATEQISFLRKLYHNKLHVSERSQRIVKQAMLTEANADYIIRAKTGYSTRIEPKIGWWVGWVELDDNVWFFAMNMDMPTSDGLGLRQAITKEVLKQEKIIP

SEQ ID NO: 43 - protein, 241 aa, Escherichia coli
KEWQENKSWNAHFTEHKSQGVVVLWNENKQQGFTNNLKRANQAFLPASTFKIPNSLIALDLGVVKDEHQVFKWDGQTRDIATWNRDHNLITAMKYSVVPVYQEFARQIGEARMSKMLHAFDYGNEDISGNVDSFWLDGGIRISATEQISFLRKLYHNKLHVSERSQRIVKQAMLTEANGDYIIRAKTGYGYDTKIGWWVGWVELDDNVWFFAMNMDMPTSDGLGLRQAITKEVLKQEKIIP

SEQ ID NO: 44 - protein, 239 aa, Escherichia coli
KEWQENKSWNAHFTEHKSQGVVVLWNENKQQGFTNNLKRANQAFLPASTFKIPNSLIALDLGVVKDEHQVFKWDGQTRDIATWNRDHNLITAMKYSVVPVHQEFARQIGEARMSKMLHAFDYGNEDISGNVDSFWLDGGIRISATEQISFLRKLYHNKLHVSERSQRIVKQAMLTEANGDYIIRAKTGYDTKIGWWVGWVELDDNVWFFAMNMDMPTSDGLGLRQAITKEVLKQEKIIP

SEQ ID NO: 45 - protein, 243 aa, Klebsiella pneumoniae
KEWQENKSWNAHFTEHKSQGVVVLWNENKQQGFTNNLKRANQAFLPASTFKIPNSLIALDLGVVKDEHQVFKWDGQTRDIAAWNRDHDLITAMKYSVVPVYQEFARQIGEARMSKMLHAFDYGNEDISGNVDSFWLDGGIRISATQQIAFLRKLYHNKLHVSERSQRIVKQAMLTEANGDYIIRAKTGYSTGIEPKIGWWVGWVELDDNVWFFAMNMDMPTSDGLGLRQAITKEVLKQEKIIP

SEQ ID NO: 46 - protein, 243 aa, Enterobacter asburiae
KEWQENKSWNAHFSEHKTQGVVVLWNENTQQGFTNDLKRANQAFLPASTFKIPNSLIALDLGVVKDEHQVFKWDGQTRDIAAWNRDHDLITAMKYSVVPVYQEFARQIGEARMSKMLHAFDYGNEDISGNLDSFWLDGGIRISATQQIAFLRKLYHNKLHVSERSQRIVKQAMLTEANADYIIRAKTGYSVRIEPKIGWWVGWIELDDNVWFFATNMDMPTAEGLGLRQTITKAVLKQEKIIP

SEQ ID NO: 47 - protein, 243 aa, Klebsiella pneumoniae; identical to SEQ ID NO: 29

SEQ ID NO: 48 - protein, 243 aa, Shewanella sp. 10A
KEWQENKSWNAHFTEHKSQGVVVLWNENKQQGFTNNLKRANQAFLPASTFKIPNSLIALDLGVVKDEHQVFKWDGQTRDIATWNRDHNLITAMKYSVVPVYQEFARQIGEARMSKMLHAFDYGNEDISGNLDTFWLDGGIRISATEQISFLRKLYHNKLHVSERSQRIVKQAMLTEANGDYIIRAKTGYSTRIEPKIGWWVGWVELDDNVWFFAMNMDMPTSDGLGLRQAITKEVLKQEKIIP

SEQ ID NO: 49 - protein, 243 aa, Shewanella sp. W17
KEWQENKSWNAHFTEHKSQGVVALWNENKQQGFTNNLKRANQAFLPASTFKIPNSLIALDLGVVKDEHQVFKWDGQTRDIATWNRDHNLITAMKYSVVPVYQEFARQIGEARMSKMLHAFDYGNEDISGNVDSFWLDGGIRISATEQISFLRKLYHNKLHVSERSQRIVKQAMLTEANSDYIIRAKTGYSTRIEPKIGWWVGWVELDDNVWFFAMNMDMPTSDGLGLRQAITKEVLKQEKIIP

SEQ ID NO: 50 - protein, 241 aa, Klebsiella pneumoniae
KEWQENKSWNAHFTEHKSQGVVVLWNENKQQGFTNNLKRANQAFLPASTFKIPNSLIALDLGVVKDEHQVFKWDGQTRDIATWNRDHNLITAMKYSVVPVYQEFARQIGEARMSKMLHAFDYGNEDISGNVDSFWLDGGIRISATEQISFLRKLYHNKLHVSERSQRIVKQAMLTEANGDYIIRAKTGYSTKPKIGWWVGWVELDDNVWFFAMNMDMPTSDGLGLRQAITKEVLKQEKIIP

SEQ ID NO: 51 - protein, 243 aa, Klebsiella pneumoniae
KEWQENKSWNAHFTEHKSQGVVVLWNENKQQGFTNNLKRANQAFLPASTFKIPNSLIALDLGVVKDEHQVFKWDGQTRDIATWNRDHNLITAMKYSVLPVYQEFARQIGEARMSKMLHAFDYGNEDISGNVDSFWLDGGIRISATEQISFLRKLYHNKLHVSERSQRIVKQAMLTEANGDYIIRAKTGYSTRIEPKIGWWVGWVELDDNVWFFAMNMDMPTSDGLGLRQAITKEVLKQEKIIP

SEQ ID NO: 52 - protein, 243 aa, Shewanella xiamenensis
KEWQENKSWNAHFTEHKSQGVVVLWNENKQQGFTNNLKRANQAFLPASTFKIPNSLIALDLGVVKDEHQVFKWDGQTRDIATWNRDHNLITAMKYSVVPVYQEFARQIGEARMSKMLHAFDYGNEDISGNVDSFWLDGGIRISATEQISFLRKLYHNKLHVSERSQRIVKQAMLTEANADYIIRAKTGYSGRIEPKFGWWVGWVELDDNVWFFAMNMDMPTSDGLGLRQAITKEVLKQEKIIP

SEQ ID NO: 53 - protein, 243 aa, Shewanella xiamenensis
REWQENKSWNVHFTEHKSQGVVVLWNENKQQGFTNNLKRANQAFLPASTFKIPNSLIALDLGVVKDEHQVFKWDGQTRDIATWNRDHNLITAMKYSVVPVYQEFARQIGEARMSKMLHAFDYGNEDISGNVDSFWLDGGIRISAIEQISFLRKLYHNKLHVSERSQRIVKQAMLTEANGDYIIRAKTGYSTRIEPKIGWWVGWVELDDNVWFFAMNMDMPTSDGLGLRQAITKEVLKQEKIIP

SEQ ID NO: 54 - protein, 243 aa, Shewanella xiamenensis
KEWQENKSWNAHFTEHKSQGVVALWNENKQQGFTNNLKRANQAFLPASTFKIPNSLIALDLGVVKDEHQVFKWDGQTRDIATWNRDHNLITAMKYSVVPVYQEFARQIGEARMSKMLHAFDYGNEDISGNVDSFWLDGGIRISAIEQISFLRKLYHNKLHVSERSQRIVKQAMLTEANGDYIIRAKTGYSTRIEPKIGWWVGWVELDDNVWFFAMNMDMPTSDGLGLRQAITKEVLKQEKIIP

SEQ ID NO: 55 - protein, 243 aa, Escherichia coli
KEWQENKSWNAHFTEHKSQGVVVLWNENKQQGFTNNLKRANQAFLPASTFKIPNSLIALDLGVVKDEHQVFKWDGQTRDIATWNRDHNLITAMKYSVVPVYQEFARQIGEARMSKMLHDFDYGNEDISGNVDSFWLDGGIRISATEQISFLRKLYHNKLHVSERSQRIVKQAMLTEANGDYIIRAKTGYSTRIEPKIGWWVGWVELDDNVWFFAMNMDMPTSDGLGLRQAITKEVLKQEKIIP

SEQ ID NO: 56 - protein, 243 aa, Shewanella sp. FDAARGOS_354
KEWQENKSWNAHFTEHKSQGVVALWNENKQQGFTNNLKRANQAFLPASTFKIPNSLIALDLGVVKDEHQVFKWDGQTRDIATWNRDHNLITAMKYSVVPVYQEFARQIGEARMSKMLHAFDYGNEDISGNVDSFWLDGGIRISATEQISFLRKLYHNKLHVSERSQRIVKQAMLTEANGDYIIRAKTGYSTRIEPKIGWWVGWVELDDNVWFFAMNMDMPTSDGLGLRQAITKEVLKQEKIIP